European Patent Application EP 4 328 316 A1, published February 28, 2024. Title: PREPARATION METHOD FOR POLYPEPTIDE. Applicant: ASYMCHEM LABORATORIES(TIANJIN) CO., LTD. The sequence listing filed with the application follows.

SEQUENCE LISTING (6 sequences)

SEQ ID NO: 1 - DNA, 411 bp, Artificial Sequence
  Sumo tag+Liraglutide precursor gene
catatgggcggcagtctgcaagatagcgaagtgaatcaagaagcgaagccagaagtgaaaccggaagttaaaccggagacccacatcaatctgaaggtgagcgacggcagcagcgagatcttcttcaagatcaagaagacgaccccgctgcgtcgtctgatggaagccttcgccaaacgccaaggcaaagaaatggacagtctgcgctttctgtacgatggtatccgcatccaagccgatcaagccccggaagatctggacatggaggacaacgacatcatcgaggcgcatcgcgaacagatcggcggccatgccgaaggcaccttcaccagcgatgttagcagctatctggaaggccaagccgccaaagaattcatcgcgtggctggttcgcggccgcggttagctcgag

SEQ ID NO: 2 - DNA, 414 bp, Artificial Sequence
  Sumo tag+Nesiritide gene
catatgggcggcagtctgcaagatagcgaagtgaatcaagaagcgaagccagaagtgaaaccggaagttaaaccggagacccacatcaatctgaaggtgagcgacggcagcagcgagatcttcttcaagatcaagaagacgaccccgctgcgtcgtctgatggaagccttcgccaaacgccaaggcaaagaaatggacagtctgcgctttctgtacgatggtatccgcatccaagccgatcaagccccggaagatctggacatggaggacaacgacatcatcgaggcgcatcgcgaacagatcggcggctctccgaaaatggttcagggttctggttgcttcggtcgtaaaatggaccgtatctcttcttcttctggtctgggttgcaaagttctgcgtcgtcactagctcgag

SEQ ID NO: 3 - DNA, 420 bp, Artificial Sequence
  Sumo tag+Teriparatide gene
catatgggcggcagtctgcaagatagcgaagtgaatcaagaagcgaagccagaagtgaaaccggaagttaaaccggagacccacatcaatctgaaggtgagcgacggcagcagcgagatcttcttcaagatcaagaagacgaccccgctgcgtcgtctgatggaagccttcgccaaacgccaaggcaaagaaatggacagtctgcgctttctgtacgatggtatccgcatccaagccgatcaagccccggaagatctggacatggaggacaacgacatcatcgaggcgcatcgcgaacagatcggcggctctgtttctgaaatccagctgatgcacaacctgggtaaacacctgaactctatggaacgtgttgaatggctgcgtaaaaaactgcaggacgttcacaacttctaactcgag

SEQ ID NO: 4 - DNA, 52 bp, Artificial Sequence
  primer Ulp1-F
gggcatatggatcttaaaaaaaagaaagaacaattggccaagaagaaacttg

SEQ ID NO: 5 - DNA, 42 bp, Artificial Sequence
  primer Ulp1-R
gggctcgaggtattttaaagcgtcggttaaaatcaaatgggc

SEQ ID NO: 6 - DNA, 699 bp, Artificial Sequence
  Ulp1 gene
gatcttaaaaaaaagaaagaacaattggccaagaagaaacttgttcctgaattaaatgaaaaagacgatgaccaagtacaaaaagctttggcatctagagaaaatactcagttaatgaatagagataatatagagataacagtacgtgattttaagaccttggcaccacgaagatggctaaatgacactatcattgagttttttatgaaatacattgaaaaatctacccctaatacagtggcgtttaattcatttttctataccaatttatcagaaaggggttatcaaggcgtccggaggtggatgaagagaaagaagacacaaattgataaacttgataaaatctttacaccaataaatttgaaccaatcccactgggcgttgggcataattgatttaaaaaagaaaactataggttacgtagattcattatcgaatggtccaaatgctatgagtttcgctatactgactgacttgcaaaaatatgttatggaggaaagtaagcatacaataggagaagactttgatttgattcatttagattgtccgcagcaaccaaatggctacgactgtggaatatatgtttgtatgaatactctctatggaagtgcagatgcgccattggattttgattataaagatgcgattaggatgagaagatttattgcccatttgattttaaccgacgctttaaaatag